European Patent Specification EP 3 966 206 B1, published August 9, 2023. Title: HETEROARYLAMINOPYRIMIDINE AMIDE AUTOPHAGY INHIBITORS AND METHODS OF USE THEREOF. Applicant: DECIPHERA PHARMACEUTICALS, LLC. The sequence listing filed with the application follows.

SEQUENCE LISTING (6 sequences)

SEQ ID NO: 1 - protein, 344 aa, Artificial Sequence
  source: /note="Description of Artificial Sequence: Synthetic polypeptide"
MSYYHHHHHHDYDIPTTENLYFQGAMDPFFMEPGRGGTETVGKFEFSRKDLIGHGAFAVVFKGRHREKHDLEVAVKCINKKNLAKSQTLLGKEIKILKELKHENIVALYDFQEMANSVYLVMEYCNGGDLADYLHAMRTLSEDTIRLFLQQIAGAMRLLHSKGIIHRDLKPQNILLSNPAGRRANPNSIRVKIADFGFARYLQSNMMAATLCGSPMYMAPEVIMSQHYDGKADLWSIGTIVYQCLTGKAPFQASSPQDLRLFYEKNKTLVPTIPRETSAPLRQLLLALLQRNHKDRMDFDEFFHHPFLDASPSVRKSPPVPVPSYPSSGSGSSSSSSSTSHLAS

SEQ ID NO: 2 - protein, 283 aa, Unknown
  source: /note="Description of Unknown: ULK1 sequence"
MEPGRGGTETVGKFEFSRKDLIGHGAFAVVFKGRHRAAHDLEVAVKCINKKNLAKSQTLLGKEIKILKELKHENIVALYDFQEMANSVYLVMEYCNGGDLADYLHAMRTLSEDTIRLFLQQIAGAMRLLHSKGIIHRDLKPQNILLSNPAGRRANPNSIRVKIADFGFARYLQSNMMAATLCGSPMYMAPEVIMSQHYDGKADLWSIGTIVYQCLTGKAPFQASSPQDLRLFYEKNKTLVPTIPRETSAPLRQLLLALLQRNHKDRMDFDEFFHHPFLDASPS

SEQ ID NO: 3 - protein, 542 aa, Artificial Sequence
  source: /note="Description of Artificial Sequence: Synthetic polypeptide"
MSPILGYWKIKGLVQPTRLLLEYLEEKYEEHLYERDEGDKWRNKKFELGLEFPNLPYYIDGDVKLTQSMAIIRYIADKHNMLGGCPKERAEISMLEGAVLDIRYGVSRIAYSKDFETLKVDFLSKLPEMLKMFEDRLCHKTYLNGDHVTHPDFMLYDALDVVLYMDPMCLDAFPKLVCFKKRIEAIPQIDKYLKSSKYIAWPLQGWQATFGGGDHPPKSDLEVLFQGPEFMEVVGDFEYSKRDLVGHGAFAVVFRGRHRQKTDWEVAIKSINKKNLSKSQILLGKEIKILKELQHENIVALYDVQELPNSVFLVMEYCNGGDLADYLQAKGTLSEDTIRVFLHQIAAAMRILHSKGIIHRDLKPQNILLSYANRRKSSVSGIRIKIADFGFARYLHSNMMAATLCGSPMYMAPEVIMSQHYDAKADLWSIGTVIYQCLVGKPPFQANSPQDLRMFYEKNRSLMPSIPRETSPYLANLLLGLLQRNQKDRMDFEAFFSHPFLEQGPVKKSCPVPVPMYSGSVSGSSCGSSPSCRFASHHHHHH

SEQ ID NO: 4 - protein, 1795 aa, Unknown
  source: /note="Description of Unknown: LRRK2 sequence"
MAPILGYWKIKGLVQPTRLLLEYLEEKYEEHLYERDEGDKWRNKKFELGLEFPNLPYYIDGDVKLTQSMAIIRYIADKHNMLGGCPKERAEISMLEGAVLDIRYGVSRIAYSKDFETLKVDFLSKLPEMLKMFEDRLCHKTYLNGDHVTHPDFMLYDALDVVLYMDPMCLDAFPKLVCFKKRIEAIPQIDKYLKSSKYIAWPLQGWQATFGGGDHPPKSDLVPRHNQTSLYKKAGTMHSDSISSLASEREYITSLDLSANELRDIDALSQKCCISVHLEHLEKLELHQNALTSFPQQLCETLKSLTHLDLHSNKFTSFPSYLLKMSCIANLDVSRNDIGPSVVLDPTVKCPTLKQFNLSYNQLSFVPENLTDVVEKLEQLILEGNKISGICSPLRLKELKILNLSKNHISSLSENFLEACPKVESFSARMNFLAAMPFLPPSMTILKLSQNKFSCIPEAILNLPHLRSLDMSSNDIQYLPGPAHWKSLNLRELLFSHNQISILDLSEKAYLWSRVEKLHLSHNKLKEIPPEIGCLENLTSLDVSYNLELRSFPNEMGKLSKIWDLPLDELHLNFDFKHIGCKAKDIIRFLQQRLKKAVPYNRMKLMIVGNTGSGKTTLLQQLMKTKKSDLGMQSATVGIDVKDWPIQIRDKRKRDLVLNVWDFAGREEFYSTHPHFMTQRALYLAVYDLSKGQAEVDAMKPWLFNIKARASSSPVILVGTHLDVSDEKQRKACMSKITKELLNKRGFPAIRDYHFVNATEESDALAKLRKTIINESLNFKIRDQLVVGQLIPDCYVELEKIILSERKNVPIEFPVIDRKRLLQLVRENQLQLDENELPHAVHFLNESGVLLHFQDPALQLSDLYFVEPKWLCKIMAQILTVKVEGCPKHPKGIISRRDVEKFLSKKRKFPKNYMSQYFKLLEKFQIALPIGEEYLLVPSSLSDHRPVIELPHCENSEIIIRLYEMPYFPMGFWSRLINRLLEISPYMLSGRERALRPNRMYWRQGIYLNWSPEAYCLVGSEVLDNHPESFLKITVPSCRKGCILLGQVVDHIDSLMEEWFPGLLEIDICGEGETLLKKWALYSFNDGEEHQKILLDDLMKKAEEGDLLVNPDQPRLTIPISQIAPDLILADLPRNIMLNNDELEFEQAPEFLLGDGSFGSVYRAAYEGEEVAVKIFNKHTSLRLLRQELVVLCHLHHPSLISLLAAGIRPRMLVMELASKGSLDRLLQQDKASLTRTLQHRIALHVADGLRYLHSAMIIYRDLKPHNVLLFTLYPNAAIIAKIADYGIAQYCCRMGIKTSEGTPGFRAPEVARGNVIYNQQADVYSFGLLLYDILTTGGRIVEGLKFPNEFDELEIQGKLPDPVKEYGCAPWPMVEKLIKQCLKENPQERPTSAQVFDILNSAELVCLTRRILLPKNVIVECMVATHHNSRNASIWLGCGHTDRGQLSFLDLNTEGYTSEEVADSRILCLALVHLPVEKESWIVSGTQSGTLLVINTEDGKKRHTLEKMTDSVTCLYCNSFSKQSKQKNFLLVGTADGKLAIFEDKTVKLKGAAPLKILNIGNVSTPLMCLSESTNSTERNVMWGGCGTKIFSFSNDFTIQKLIETRTSQLFSYAAFSDSNIITVVVDTALYIAKQNSPVVEVWDKKTEKLCGLIDCVHFLREVMVKENKESKHKMSYSGRVKTLCLQKNTALWIGTGGGHILLLDLSTRRLIRVIYNFCNSVRVMMTAQLGSLKNVMLVLGYNRKNTEGTQKQKEIQSCLTVWDINLPHEVQNLEKHIEVRKELAEKMRRTSVE

SEQ ID NO: 5 - protein, 16 aa, Artificial Sequence
  source: /note="Description of Artificial Sequence: Synthetic peptide"
YANWLAASIYLDGKKK

SEQ ID NO: 6 - protein, 15 aa, Artificial Sequence
  source: /note="Description of Artificial Sequence: Synthetic peptide"
RLGRDKYKTLRQIRQ